European Patent Application EP 4 772 627 A1, published July 8, 2026. Title: tRNA及其生物合成方法. Applicant: 吉林凯莱英医药化学有限公司. The sequence listing filed with the application follows.

SEQUENCE LISTING (38 sequences)

SEQ ID NO: 1 - protein, 375 aa, Escherichia phage JN02
HMEKLYYNLLSLCKSSSDRKFFYSDDVSPIGKKYRIFSYNFASYSDWLLPDALECRGIMFEMDGETPVRIASRPMEKFFNLNENPFTLSINLDDVKYLMTKEDGSLVSTYLDGGTVRFKSKGSIKSDQAVSATSILLDIDHKNLADRLLELCNDGFTANFEYVAPTNKIVLTYPEKRLILLNIRDNNTGEYIEYDDIYLDPVFRKYLVDRFEVPEGDWTSDVKSSTNIEGYVAVMKDGSHFKLKTDWYVALHTTRDSISSPEKLFLAIVNGASDDLKAMYADDEFSFKKVELFEKAYLDFLDRSFYICLDTYDKHKGKDRKTYAIEAQAVCKGAQTPWLFGIIMNLYQGGSKEQMMTALESVFIKNHKNFIPEGY

SEQ ID NO: 2 - protein, 374 aa, Bacteriophage AR1
MQELFNNLMELCKDSQRKFFYSDDVSASGRTYRIFSYNYASYSDWLLPDALECRGIMFEMDGEKPVRIASRPMEKFFNLNENPFTMNIDLNDVDYILTKEDGSLVSTYLDGDEILFKSKGSIKSEQALMANGILMNINHHQLRDRLKELAEDGFTANFEFVAPTNRIVLAYQEMKIILLNIRENETGEYISYDDIYKDAALRPYLVERYEIDSPKWVEEAKNAENIEGYVAVMKDGSHFKIKSDWYVSLHSTKSSLDNPEKLFKTIIDGASDDLKAMYADDEYSYRKIEAFETTYLKYLDRALFLVLDCHNKHCGKDRKTYAMEAQGVAKGAGMDHLFGIIMSLYQGYDSQEKVMCEIEQNFLKNYKKFIPEGY

SEQ ID NO: 3 - protein, 335 aa, Bacteriophage dhaeg
MFKKYSSLENHYNSKFIEKLRTNGLTGGEWVAREKIHGTNFSLIIERDAVTCAKRTGPILPAEDFYGYEIVLKNYADSIKSIQDIMETSAAVSYQVFGEFAGTGIQKNVDYGDKDFYVFDIIVTTESGDVTYVDDYMMESFCKTFKFKMAPLLGRGKFEDLIKLPNDLDSVLPDYNFTVDNVGLAEANAHVWNAEAKGEVFTAEGYVLKPCYPLWLPNGNRVAIKCKNSKFSEKKKTDKPIKVAVVLSQDDLDLLQQFTDYVTVNRINNVISKIGEVSPKDFGKVMGLTVQDILEEAAREELELTDAENPVEVKKQLIECVKDTLRAVWIELVSK

SEQ ID NO: 4 - protein, 335 aa, Vibrio phage
MSFVKYTSLENSYRQAFVDKCDMLGVREWVALEKIHGANFSFIVEFKPNEAQDGAEFTVTPAKRTSTIGANVMGDYDFYGCTSVVEAHTAKMEAISNWLWARGIINVGETIIVYGELAGKGVQKEVNYGDKDFWAYDILLPETGKFLDWDVVLEACEFAKVKTTHEIARGTLDELLRIDPLFRSFHTPADVDGDNVAEGFVVKQLRNEKRLHNGSRAILKVKNDKFKEKKNKAGKTPRAAVVLTEEQEKLHAAFSCYLTENRLRNVLSKLETVTQKQFGMISGLFIKDAKDEFERDELNETAIARDDWDVIKRSLTNIANEILRKNWLDILDGNF

SEQ ID NO: 5 - protein, 379 aa, Archaea
MVSSVYKEILVKLGLTEDRIETLEMKGGIIEDEFDGIRYVRFKDSAGKLRRGTVVIDEEYVIPGFPHIKRIINLRSGIRRIFKRGEFYVEEKVDGYNVRVVMYKGKMLGITRGGFICPFTTERIPDFVPQEFFKDNPNLILVGEMAGPESPYLVEGPPYVKEDIQFFLFDVQEIKTGRSLPVEERLKIAEEYGINHVEVFGKYTKDDVDELYQLIERLSKEGREGIIMKSPDMKKIVKYVTPYANINDIKIGARVFYELPPGYFTSRISRLAFYLAEKRIKGEEFERVAKELGSALLQPFVESIFDVEQEEDIHELFKVRVKRIETAYKMVTHFEKLGLKIEIVDIEEIKDGWRITFKRLYPDATNEIRELIGGKAFVD

SEQ ID NO: 6 - protein, 342 aa, fungus Deinococcus radiodurans
MAERQVIKERAQLFPHPNAERLELCKVGTFQLVVRKGEYRDGDPIVIAPEKAVLPPQLAGLYTNADTGASYLHGAEKNRVGSVRLRGEVSQGVILPLDGLEDAPFGEDLAERLGITFWEPPVPVSMAGEVEPRPPAQHYKHHDVEQFGIYVSEFASGEEVMVTEKLHGTQGVYFRTAEGRWLVTSKGLSRGGLTLREAASNVYWQAARNSNLFAEADAAFSGGEVQIFGEVVPVQKGFSYGQHKPTVFVFKVVYDGLRLPRRDWPQWVLDHAVPVLYEGPFDEATVRKLRGGLETVSGKGLHIREGVVVAPKVPRFAADGSDLSVKLISDAYAKKETGEEYS

SEQ ID NO: 7 - protein, 400 aa, Trypanosoma brucei brucei
MVGGDGSIFERYTEIDNSNERRINALKGCGMFEDEWIATEKVHGANFGIYSIEGEKMIRYAKRSGIMPPNEHFFGYHILIPELQRYVTSIREMLCEKQKKKLHVVLINGELFGGKYDHPSVPKTRKTVMVAGKPRTISAVQTDSFPQYSPDLHFYAFDIKYKETEGGDYTTLVYDEAIELFQRVPGLLYARAVIRGPMSKVAAFDVERFVTTIPPLVGMGNYPLTGNWAEGLVVKHSRLGMAGFDPKGPTVLKFKCTAFQEISTDRAQGPRVDEMRNVRRDSINRAGVQLPDLESIVQDPIQLEASKLLLNHVCENRLKNVLSKIGTEPFEKEEMTPDQLATLLAKDALKDFLKDTEPSIVNIPVLIRKDLTRYVIFESRRLVCSQWKDILKRQSPDFSE

SEQ ID NO: 8 - protein, 382 aa, Acidobacteria bacterium
MKQMYDNLKALTQKNDMFFSSIQTTPSNKPVEIFSYHIASYSDWLEPDAIECRGIMFDITDKENPVILSRPMEKFFNLGENPLALPEDVLPLVKTIEEKRDGSLISTYLDDGKLYTKSKGSLYSDQANDSNRFLMRSENKDFKQALKTLAELGYTANMEYTSPKNQIVLKYEKQELIVLNIRNTETGDYLTLDDLAELDAENPEHTIYTHIAERFVDYEEVDGMSDEDVERIRDMKGIEGYVLVGQNQRVKLKTDWYVNLHRLKDNINNNRRLVESVVESRTDDLRQLFEHDQGSIDKIKEFEQYVLSKIKSCLAEVRTVYERVKHLDRKHYAINAQRYVDYTPLFSVIMRQFDDYNEENVVENIKQIALKNVDDFIPMHYK

SEQ ID NO: 9 - protein, 428 aa, fungus Magnaporthe grisea
MEGDSPVVAVTSPTIPTDSTLAVSPTAEKAASTESFSAPAVRKLVTLRRISRIRPVKNAKLPKSKYVAITVDGWEVVVNAKRDQRRFREGQLVVFFQIDSFVPENDGNFWEEMSTSAELFQERRGFRIGTLRIGESSLISQGRVFHLGEYPRVEEVVAELQKVHGDKDGLEVAMQRSFDDVLGVVKWDVPEEHKGAHYGPPPPMIPRTALNRIQDVTQQLWERHAATRVQITEKLDSCPISIYFVRNDSPFAKCLPALHDFAGKPDAQRRQQQLCVFPHGRVGVCANRLEYVCAPGQRFWAVVERLGIPGRLAREGRTAVVQGELVAPDRGGPGGFYAFSLWTEGGKHGGFDGEETQRAALRRMGVPLVPLVGYRAIGEFASSTGEMLAKADGRGFRGQLREGFVLKNVKENIWVKVISNAWLEWYEE

SEQ ID NO: 10 - protein, 339 aa, Klebsiella phage KP15
MFKKYSSLTNHYEGKFINGVIMNGLTGGVWVAREKIHGANFSFITDDGITVTPAKRTDVVKPAEDFYGCSAVVAKYSPGIRKMWETLKKTGTYDDLVIQVYGEFAGRGVQKDVDYGEKDFYVFDIRVNGEFLPDNLCSLISRSHGLKMAPLLGYGTFEEIKELPITFESVVNKANSGIGSDNTVYGEFVYPIMDVEEGNIAEGFVMKPVSPAFMPNGERVAIKCKTTKFTEKKAKKATRFNAPVSLSEKDKNQLDEFVCYLTENRVKNVLSKLDLASITAKDFGRIMGLTVQDAIEEISRNHGPFIEQFEDPAMAKKLFVTEAQNMIRPVWGKILNHEF

SEQ ID NO: 11 - protein, 381 aa, Vibrio phage
MTTQELYNHLMTLTDDAEGKFFFADHISPLGEKLRVFSYHIASYSDWLLPGALEARGIMFQLDEQDKMVRIVSRPMEKFFNLNENPFTMDLDLTTTVQLMDKADGSLISTYLTGENFALKSKTSIFSEQAVAANRYIKLPENRDLWEFCDDLTQAGCTVNMEWCAPNNRIVLEYPEAKLVILNIRDNETGDYVSFDDIPLPALMRVKKWLVDEYDPETAHADDFVEKLRATKGIEGMILRLANGQSVKIKTQWYVDLHSQKDSVNVPKKLVTTILNNNHDDLYALFADDKPTIDRIREFDSHVSKTVSASFHAVSQFYVKNRHMSRKDYAIAGQKTLKPWEFGVAMIAYQNQTVEGVYEALVGAYLKRPELLIPEKYLNEA

SEQ ID NO: 12 - protein, 334 aa, Bacteriophage
MFKKYSSLENHYNSKFIEKLYSLGLTGGEWVAREKIHGTNFSLIIERDKVTCAKRTGPILPAEDFFGYEIILKNYADSIKAVQDIMETSAVVSYQVFGEFAGPGIQKNVDYCDKDFYVFDIIVTTESGDVTYVDDYMMESFCNTFKFKMAPLLGRGKFEELIKLPNDLDSVVQDYNFTVDHAGLVDANKCVWNAEAKGEVFTAEGYVLKPCYPSWLRNGNRVAIKCKNSKFSEKKKSDKPIKAKVELSEADNKLVGILACYVTLNRVNNVISKIGEIGPKDFGKVMGLTVQDILEETSREGITLTQADNPSLIKKELVKMVQDVLRPAWIELVS

SEQ ID NO: 13 - protein, 327 aa, bacteria
MSFVKYTSLENSYRQAFVDKCDMLGVRDWVALEKIHGANFSFIVEFDGGYTVTPAKRTSIIGATATGDYDFYGCTSVVEAHKEKVELVANFLWLNEYINLYEPIIIYGELAGKGIQKEVNYGDKDFWAFDIFLPQREEFVDWDTCVAAFTNAEIKYTKELARGTLDELLRIDPLFKSLHTPAEHEGDNVAEGFVVKQLHSEKRLQSGSRAILKVKNEKFKEKKKKEGKTPTKLVLTPEQEKLHAEFSCYLTENRLKNVLSKLGTVNQKQFGMISGLFVKDAKDEFERDELNEVAIDRDDWNAIRRSLTNIANEILRKNWLNILDGNF

SEQ ID NO: 14 - protein, 381 aa, Vibrio phage phi-ST2
MNVQELYKNLMSLADDAEGKFFFADHLSPLGEKFRVFSYHIASYSDWLLPGALEARGIMFQLDDNDEMIRIVSRPMEKFFNLNENPFTMELDLTTTVQLMDKADGSLISTYLSGENFALKSKTSIFSEQAVAANRYIKKPENRDLWEFCDDCTQAGLTVNMEWCAPNNRIVLEYPEAKLVILNIRDNETGDYVSFDDIPQSALMRVKQWLVDEYDPATAHEPDFVEKLRDTKGIEGMILRLANGQSVKIKTQWYVDLHSQKDSVNVPKKLVTTILNGNHDDLYALFADDKPTIERIREFDSHVTKTLTNSFNAVRQFYARNRHLARKDYAIAGQKVLKPWEFGVAMIAYQKQTVEGVYESLVTAYLKRPELAIPEKYLNGV

SEQ ID NO: 15 - protein, 335 aa, Vibrio phage JN02
MFKKYSSLENHYNSKFIEKLYTNGLTTGVWVAREKIHGTNFSLIIERDNVTCAKRTGPILPAEDFYGYEIVLKKYDKAIKAVQEVMESISTSVPVSYQVFGEFAGGGIQKGVDYGEKDFYVFDIIINTESDDTYYMSDYEMQDFCNTFGFKMAPMLGRGTFDSLIMIPNDLDSVLAAYNSTASEDLVEANNCVFDANVIGDNTAEGYVLKPCFPKWLSNGTRVAIKCKNSKFSEKKKSDKPVKTQVPLTEIDKNLLDVLACYVTLNRVNNVISKIGTVTPKDFGKVMGLTVQDILEETSREGIVLTSSDNPNLVKKELVRMVQDVLRPAWIELVS

SEQ ID NO: 16 - protein, 334 aa, Vibrio phage JS98
MFKKYSSLENHYNSKFIEKLRTNGLTGGEWVAREKIHGTNFSLIIERDAVTCAKRTGPILPAEDFYGYEIVLKNYADSIKSVQHLIESINYQSYQIYGELAGPGIQKNVDYGDKDFYVFDIRVTKEDGTESVLTDTLMEAFCIIHKFKVAPCLATGSFEDLIKLPNDFDSVIPDYNFAVDNAGLTIANSTDFIPKVEGKVFTAEGFVLKPDIPTWLPNGNRVAIKCKNSKFSEKKKSDKPIKAAVVLSQDDMDLMWQFTDYVTVNRINNVISKIGEVSKKDFGKVMGLTVQDILEEAAREELELTDAENPVEVKKQLVECVKDTLRAVWIELVS

SEQ ID NO: 17 - protein, 416 aa, Trypanosoma brucei gambiense
MLRCLGVRHFRRTPLLFVGGDGSIFERYTEIDNSNERRINALKGCGMFEDEWIATEKVHGANFGIYSIEGEKMIRYAKRSGIMPPNEHFFGYHILIPELQRYVTSIREMLCEKQKKKLHVVLINGELFGGKYDHPSVPKTRKTVMVAGKPRTISAVQTDSFPQYSPDLHFYAFDIKYKETEGGDYTTLVYDEAIELFQRVPGLLYARAVIRGPMSKVAAFDVERFVTTIPPLVGMGNYPLTGNWAEGLVVKHSRLGMAGFDPKGPTVLKFKCTAFQEISTDRAQGPRVDEMRNVRRDSINRAGVQLPDLESIVQDPIQLEASKLLLNHVCENRLKNVLSKIGTEPFEKEEMTPDQLATLLAKDAMKDFLKDTEPSIVNIPVLIRKDLTRYVIFESRRLVCSQWKDILKRQSPDFSE

SEQ ID NO: 18 - protein, 372 aa, Bacteriophage RB69
MEKLYYNLLSLCKSSSDRKFFYSDDVSPIGKKYRIFSYNFASYSDWLLPDALECRGIMFEMDGETPLRIASRPMEKFFNLNENPFTLSIDLNDVKYLMTKEDGSLVSTYLDGNMVRFKGSIKSDQAASATSILLDINHKDLADRLLELCNDGFTANFEYVAPSNKIVLTYPEKRLILLNIRDNNTGKYIEYDDIYLDPVFRKYLVDRFEAPEGDWVPGVKSSTNIEGYVAVMKDGSHFKLKTDWYVALHTTRDSISSPEKLFLAIMNGASDDLKAMYADDEFSFKKVELFEKAYLDFLDRSFYICLDAYDKHKGKDRKTYAIEAQAICKGAQSPWLFGIIMNLYQGGSKEQMMTALESVFIKNHKNFIPEGY

SEQ ID NO: 19 - protein, 374 aa, Bacteriophage
MQELFNNLMELCKDSQRKFFYSDDVSASGRTYRIFSYNYASYSDWLLPDALECRGIMFEMDGEKPVRIASRPMEKFFNLNENPFTMNIDLNDVDYILTKEDGSLVSTYLDGDEILFKSKGSIKSEQALMANGILMNINHHRLRDRLKELAEDGFTANFEFVAPTNRIVLAYQEMKIILLNVRENETGEYISYDDIYKDATLRPYLVERYEIDSPKWIEEAKNAENIEGYVAVMKDGSHFKIKSDWYVSLHSTKSSLDNPEKLFKTIIDGASDDLKAMYADDEYSYRKIEAFETTYLKYLDRALFLVLDCHNKHCGKDRKTYAMEAQGVAKGAGMDHLFGIIMSLYQGYDSQEKVMCEIEQNFLKNYKKFIPEGY

SEQ ID NO: 20 - protein, 381 aa, bacterial
MNSMNSDIPFDLIQERTGVPSSRLKVAFARGSLRLLESAGMQALLFKKPLGDLEAGTVIYLGDETEVIRGFPKIRRTLLLSPTIQEHFRDRVAVEEKMNGYNVRIACLSSGETVALTRGGHVCPFTTRKAQELLDLSEFFREHPDLVICGEMIGRDNPYVSQDYPEVGPLGFRVFDLREKNTNRPLPVEERRALLDSYGLPNVRLFGVYPIEEAASEVADIIRALGMAGREGVVMKDPSMEVPPLKYTSSQAHARELAYAFSYPFDFGRPFFFSRVIREGFQAYELDESDDETRERARRLGEAIIYPMLERIKSISAGEAAYEDTVIDVEDREAAEEFIRHLVRLGVSATLADYRDGRATIRRFYQSTTDRINNYLKGGLY

SEQ ID NO: 21 - protein, 383 aa, Klebsiella phage KP179
MLELYKNLMNLCESSEVAKFFYKDFTGPMDGKFRVFSYHYASYSEWLKPDALECRGIMFEMDGDTPIRIASRPMEKFFNLNENPLTMGIDISDVEYIMDKADGSLVSSYVDDGYLYLKSKTSLYSDQARQASALLNSEEYSSLHQVILELTLDGYTVNMEFVSPNNRVVLAYQEPQLFVLNVRNNTTGEYIKYDDLYANAKIRPYLINAYGISDPTTWVEGVRELEGVEGYIAVLNTGQRFKVKTEWYSALHHTKDSITSNERLFASVVSANSDDLRSLFAGDEYAIKKISAFEQAYLDYLGKSLELCQSFYDEYRGRARKDYAIAAQKATVNQRHLFGVIMNMYEGTVDVDKLLKDLERVFLKYWAGYVPKEYEKEIELSEE

SEQ ID NO: 22 - protein, 379 aa, Vibrio phage nt-1 rnlA
MNELYNNLMTLAESAEGKFFFADHLSPQGEKFRVFSYHIASYSDWLLPDALEARGIMFQLDENDEMIRIVSRPMEKFFNLGENPFTMDLDLTTTVQLMDKADGSLISTYLTGDNFALKSKTSIYSEQAVAANRYIKHVDNRDLWEFCDDCAAQNFTVNMEWCAPNNRIVLEYTEPKLIILNIRDNETGQYVSFDDIPIGALTRIKKWLVDEYDPMTAHVDDFVETLKAKKGIEGMILRLASGQSVKIKTTWYVDLHAQKDSVNSPKKLVTTILNKNHDDLYALFADDKPTIERIREFDDHVSKKVVESFHAVSQYYTKNRHLSRKDFAIAGQKALKPWEFGVAMIAYQNQTVEGVVTMLINAYLKRPELLIPEKYLSEV

SEQ ID NO: 23 - protein, 335 aa, Vibrio phage phi-ST2
MSFVKYTSLENSYRQAFVDKCDMLGVKEWVALEKIHGANFSFIVEFKPSTEEVPGEMSVTPAKRTSTIGANAMGDYDFYGCTSVVEAHIEKMQDISNWLFANDFIKNDETIIVYGELAGKGIQKEVNYGDKDFWAYDILCPETGEFLDWDVVLKACKFAGVKTTHEIARGTLDELLKIDPLFRSFHTPADVDSENVAEGFVVKQLKAEKRLHNGSRAILKVKNEKFKEKKNKQGKTPRAKVVLTEEQEKLHAAFSCYLTENRLRNVLSKIGKVEAKQFGMVSGLFVKDAKDEFERDERDEVAIPRDDWDVIKRSLVNVANEILRKNWLNIVDGTF

SEQ ID NO: 24 - RNA, 37 nt, synthetic construct
  source 1..37: mol_type = other RNA; note; note (original language) = 底物1
gtgtccctgcggcaatggatagccgattggacttcaa

SEQ ID NO: 25 - RNA, 36 nt, synthetic construct
  source 1..36: mol_type = other RNA; note; note (original language) = 底物2
attcaaaggttccgggttcgagtcccgggggacgcg

SEQ ID NO: 26 - RNA, 37 nt, synthetic construct; identical to SEQ ID NO: 24
  source 1..37: mol_type = other RNA; note; note (original language) = 底物3

SEQ ID NO: 27 - RNA, 36 nt, synthetic construct; identical to SEQ ID NO: 25
  source 1..36: mol_type = other RNA; note; note (original language) = 底物4

SEQ ID NO: 28 - RNA, 37 nt, synthetic construct
  source 1..37: mol_type = other RNA; note; note (original language) = 底物5
gcgaccttagctcagttggtagagcggaggactccag

SEQ ID NO: 29 - RNA, 38 nt, synthetic construct
  source 1..38: mol_type = other RNA; note; note (original language) = 底物6
atccttaggtcactggttcgaatccggtaggtcgcacc

SEQ ID NO: 30 - RNA, 37 nt, synthetic construct; identical to SEQ ID NO: 28
  source 1..37: mol_type = other RNA; note; note (original language) = 底物7

SEQ ID NO: 31 - RNA, 38 nt, synthetic construct; identical to SEQ ID NO: 29
  source 1..38: mol_type = other RNA; note; note (original language) = 底物8

SEQ ID NO: 32 - RNA, 40 nt, synthetic construct
  source 1..40: mol_type = other RNA; note; note (original language) = 底物9
gtgtccctgcggcaatggatagccgattggacttcaaatt

SEQ ID NO: 33 - RNA, 33 nt, synthetic construct
  source 1..33: mol_type = other RNA; note; note (original language) = 底物10
caaaggttccgggttcgagtcccgggggacgcg

SEQ ID NO: 34 - RNA, 40 nt, synthetic construct; identical to SEQ ID NO: 32
  source 1..40: mol_type = other RNA; note; note (original language) = 底物11

SEQ ID NO: 35 - RNA, 33 nt, synthetic construct; identical to SEQ ID NO: 33
  source 1..33: mol_type = other RNA; note; note (original language) = 底物12

SEQ ID NO: 36 - RNA, 40 nt, synthetic construct; identical to SEQ ID NO: 32
  source 1..40: mol_type = other RNA; note; note (original language) = 底物13

SEQ ID NO: 37 - RNA, 19 nt, synthetic construct
  source 1..19: mol_type = other RNA; note; note (original language) = 底物14
attcaaaggttccgggttc

SEQ ID NO: 38 - RNA, 17 nt, synthetic construct
  source 1..17: mol_type = other RNA; note; note (original language) = 底物15
gagtcccgggggacgcg